European Patent Specification EP 3 802 873 B1, published August 2, 2023. Title: METHOD FOR DETECTING A SINGLE NUCLEOTIDE POLYMORPHISM (SNP). Applicant: Imperial College of Science, Technology and Medicine. The sequence listing filed with the application follows.

SEQUENCE LISTING (102 sequences)

SEQ ID NO: 1 - DNA, 40 bp, Artificial Sequence
  Primer
tacatagctgatgatcttatgatcatcgtatgaaagcatg

SEQ ID NO: 2 - DNA, 49 bp, Artificial Sequence
  Primer
atgttgcttttgataataaaatttatgctaataaggcatatggaaattg

SEQ ID NO: 3 - DNA, 28 bp, Artificial Sequence
  Primer
tgtgttgcttttgataataaaatttatg

SEQ ID NO: 4 - DNA, 23 bp, Artificial Sequence
  Primer
cacacatagctgatgatctaggg

SEQ ID NO: 5 - DNA, 23 bp, Artificial Sequence
  Primer
ctattataccgaatgtagaagca

SEQ ID NO: 6 - DNA, 18 bp, Artificial Sequence
  Primer
tgctcctgaacttctagc

SEQ ID NO: 7 - DNA, 20 bp, Artificial Sequence
  Primer
tcaaaggtgccacctctacc

SEQ ID NO: 8 - DNA, 25 bp, Artificial Sequence
  Primer
ggtggaactaatggtgagagattaa

SEQ ID NO: 9 - DNA, 46 bp, Artificial Sequence
  Primer
gtaagaaattattcaatacagattagatattagtcaacaatgctgg

SEQ ID NO: 10 - DNA, 38 bp, Artificial Sequence
  Primer
cacgtttttggtggtaaaaacgatcatacacctcagtt

SEQ ID NO: 11 - DNA, 25 bp, Artificial Sequence
  Primer
atacgtttttggtggtaataactat

SEQ ID NO: 12 - DNA, 26 bp, Artificial Sequence
  Primer
ataagaaattattcaatacagcactt

SEQ ID NO: 13 - DNA, 25 bp, Artificial Sequence
  Primer
ggtgtagaatatttaaattcgatgg

SEQ ID NO: 14 - DNA, 23 bp, Artificial Sequence
  Primer
ttgaaacataccatacatctctt

SEQ ID NO: 15 - DNA, 25 bp, Artificial Sequence
  Primer
tggtagacataggtgtacacatacg

SEQ ID NO: 16 - DNA, 19 bp, Artificial Sequence
  Primer
attataaggctttatttga

SEQ ID NO: 17 - DNA, 44 bp, Artificial Sequence
  Primer
gtaccatttgacgtaacactaagagatgtatggtatgtttcaag

SEQ ID NO: 18 - DNA, 43 bp, Artificial Sequence
  Primer
caatttattgtattgggggatcatatgcttctacattcggtat

SEQ ID NO: 19 - DNA, 25 bp, Artificial Sequence
  Primer
tagaatttattgtattgggggatat

SEQ ID NO: 20 - DNA, 22 bp, Artificial Sequence
  Primer
ctaccatttgacgtaacaccac

SEQ ID NO: 21 - DNA, 20 bp, Artificial Sequence
  Primer
aactgaggtgtatgatcgtt

SEQ ID NO: 22 - DNA, 18 bp, Artificial Sequence
  Primer
acccatgctttcatacga

SEQ ID NO: 23 - DNA, 21 bp, Artificial Sequence
  Primer
ttatttcttctaggtatattt

SEQ ID NO: 24 - DNA, 17 bp, Artificial Sequence
  Primer
atgatggctcttctatt

SEQ ID NO: 25 - DNA, 40 bp, Artificial Sequence; identical to SEQ ID NO: 1
  Primer

SEQ ID NO: 26 - DNA, 49 bp, Artificial Sequence; identical to SEQ ID NO: 2
  Primer

SEQ ID NO: 27 - DNA, 28 bp, Artificial Sequence
  Primer
tgtgttgcttttgataataaaatttatg

SEQ ID NO: 28 - DNA, 23 bp, Artificial Sequence
  Primer
cacacatagctgatgatctaggg

SEQ ID NO: 29 - DNA, 40 bp, Artificial Sequence
  Primer
cacatagctgatgatcttatgatcatcgtatgaaagcatg

SEQ ID NO: 30 - DNA, 49 bp, Artificial Sequence
  Primer
gtgttgcttttgataataaaatttatgctaataaggcatatggaaattg

SEQ ID NO: 31 - DNA, 35 bp, Artificial Sequence
  Primer
gtatgttgcttttgataataaaatttatgtcattg

SEQ ID NO: 32 - DNA, 22 bp, Artificial Sequence
  Primer
atacatagctgatgatctaggg

SEQ ID NO: 33 - DNA, 23 bp, Artificial Sequence
  Primer
ctattataccgaatgtagaagca

SEQ ID NO: 34 - DNA, 18 bp, Artificial Sequence
  Primer
tgctcctgaacttctagc

SEQ ID NO: 35 - DNA, 20 bp, Artificial Sequence
  Primer
tcaaaggtgccacctctacc

SEQ ID NO: 36 - DNA, 25 bp, Artificial Sequence
  Primer
ggtggaactaatggtgagagattaa

SEQ ID NO: 37 - DNA, 46 bp, Artificial Sequence; identical to SEQ ID NO: 9
  Primer

SEQ ID NO: 38 - DNA, 38 bp, Artificial Sequence; identical to SEQ ID NO: 10
  Primer

SEQ ID NO: 39 - DNA, 25 bp, Artificial Sequence
  Primer
atacgtttttggtggtaataactat

SEQ ID NO: 40 - DNA, 26 bp, Artificial Sequence
  Primer
ataagaaattattcaatacagcactt

SEQ ID NO: 41 - DNA, 46 bp, Artificial Sequence
  Primer
ataagaaattattcaatacagattagatattagtcaacaatgctgg

SEQ ID NO: 42 - DNA, 38 bp, Artificial Sequence
  Primer
tacgtttttggtggtaaaaacgatcatacacctcagtt

SEQ ID NO: 43 - DNA, 26 bp, Artificial Sequence
  Primer
tacacgtttttggtggtaataactat

SEQ ID NO: 44 - DNA, 27 bp, Artificial Sequence
  Primer
tgtaagaaattattcaatacagcactt

SEQ ID NO: 45 - DNA, 25 bp, Artificial Sequence
  Primer
ggtgtagaatatttaaattcgatgg

SEQ ID NO: 46 - DNA, 23 bp, Artificial Sequence
  Primer
ttgaaacataccatacatctctt

SEQ ID NO: 47 - DNA, 25 bp, Artificial Sequence
  Primer
tggtagacataggtgtacacatacg

SEQ ID NO: 48 - DNA, 19 bp, Artificial Sequence
  Primer
attataaggctttatttga

SEQ ID NO: 49 - DNA, 44 bp, Artificial Sequence; identical to SEQ ID NO: 17
  Primer

SEQ ID NO: 50 - DNA, 43 bp, Artificial Sequence; identical to SEQ ID NO: 18
  Primer

SEQ ID NO: 51 - DNA, 25 bp, Artificial Sequence
  Primer
tagaatttattgtattgggggatat

SEQ ID NO: 52 - DNA, 22 bp, Artificial Sequence
  Primer
ctaccatttgacgtaacaccac

SEQ ID NO: 53 - DNA, 42 bp, Artificial Sequence
  Primer
ctaccatttgacgtaactaagagatgtatggtatgtttcaag

SEQ ID NO: 54 - DNA, 44 bp, Artificial Sequence
  Primer
agaatttattgtattgggggatcatatgcttctacattcggtat

SEQ ID NO: 55 - DNA, 25 bp, Artificial Sequence
  Primer
tacaatttattgtattgggggatat

SEQ ID NO: 56 - DNA, 23 bp, Artificial Sequence
  Primer
tgtaccatttgacgtaacaccac

SEQ ID NO: 57 - DNA, 20 bp, Artificial Sequence
  Primer
aactgaggtgtatgatcgtt

SEQ ID NO: 58 - DNA, 18 bp, Artificial Sequence
  Primer
acccatgctttcatacga

SEQ ID NO: 59 - DNA, 21 bp, Artificial Sequence
  Primer
ttatttcttctaggtatattt

SEQ ID NO: 60 - DNA, 17 bp, Artificial Sequence
  Primer
atgatggctcttctatt

SEQ ID NO: 61 - DNA, 23 bp, Artificial Sequence
  Primer
ctattataccgaatgtagaagca

SEQ ID NO: 62 - DNA, 18 bp, Artificial Sequence
  Primer
tgctcctgaacttctagc

SEQ ID NO: 63 - DNA, 20 bp, Artificial Sequence
  Primer
tcaaaggtgccacctctacc

SEQ ID NO: 64 - DNA, 25 bp, Artificial Sequence
  Primer
ggtggaactaatggtgagagattaa

SEQ ID NO: 65 - DNA, 40 bp, Artificial Sequence; identical to SEQ ID NO: 29
  Primer

SEQ ID NO: 66 - DNA, 49 bp, Artificial Sequence; identical to SEQ ID NO: 30
  Primer

SEQ ID NO: 67 - DNA, 40 bp, Artificial Sequence; identical to SEQ ID NO: 1
  Primer

SEQ ID NO: 68 - DNA, 49 bp, Artificial Sequence; identical to SEQ ID NO: 2
  Primer

SEQ ID NO: 69 - DNA, 35 bp, Artificial Sequence; identical to SEQ ID NO: 31
  Primer

SEQ ID NO: 70 - DNA, 22 bp, Artificial Sequence
  Primer
atacatagctgatgatctaggg

SEQ ID NO: 71 - DNA, 28 bp, Artificial Sequence
  Primer
tgtgttgcttttgataataaaatttatg

SEQ ID NO: 72 - DNA, 23 bp, Artificial Sequence
  Primer
cacacatagctgatgatctaggg

SEQ ID NO: 73 - DNA, 25 bp, Artificial Sequence
  Primer
ggtgtagaatatttaaattcgatgg

SEQ ID NO: 74 - DNA, 23 bp, Artificial Sequence
  Primer
ttgaaacataccatacatctctt

SEQ ID NO: 75 - DNA, 25 bp, Artificial Sequence
  Primer
tggtagacataggtgtacacatacg

SEQ ID NO: 76 - DNA, 19 bp, Artificial Sequence
  Primer
attataaggctttatttga

SEQ ID NO: 77 - DNA, 46 bp, Artificial Sequence; identical to SEQ ID NO: 41
  Primer

SEQ ID NO: 78 - DNA, 38 bp, Artificial Sequence; identical to SEQ ID NO: 42
  Primer

SEQ ID NO: 79 - DNA, 46 bp, Artificial Sequence; identical to SEQ ID NO: 9
  Primer

SEQ ID NO: 80 - DNA, 38 bp, Artificial Sequence; identical to SEQ ID NO: 10
  Primer

SEQ ID NO: 81 - DNA, 26 bp, Artificial Sequence
  Primer
tacacgtttttggtggtaataactat

SEQ ID NO: 82 - DNA, 27 bp, Artificial Sequence
  Primer
tgtaagaaattattcaatacagcactt

SEQ ID NO: 83 - DNA, 25 bp, Artificial Sequence
  Primer
atacgtttttggtggtaataactat

SEQ ID NO: 84 - DNA, 26 bp, Artificial Sequence
  Primer
ataagaaattattcaatacagcactt

SEQ ID NO: 85 - DNA, 20 bp, Artificial Sequence
  Primer
aactgaggtgtatgatcgtt

SEQ ID NO: 86 - DNA, 18 bp, Artificial Sequence
  Primer
acccatgctttcatacga

SEQ ID NO: 87 - DNA, 21 bp, Artificial Sequence
  Primer
ttatttcttctaggtatattt

SEQ ID NO: 88 - DNA, 17 bp, Artificial Sequence
  Primer
atgatggctcttctatt

SEQ ID NO: 89 - DNA, 44 bp, Artificial Sequence
  Primer
ctaccatttgacgtaacactaagagatgtatggtatgtttcaag

SEQ ID NO: 90 - DNA, 43 bp, Artificial Sequence
  Primer
gaatttattgtattgggggatcatatgcttctacattcggtat

SEQ ID NO: 91 - DNA, 44 bp, Artificial Sequence; identical to SEQ ID NO: 54
  Primer

SEQ ID NO: 92 - DNA, 44 bp, Artificial Sequence; identical to SEQ ID NO: 17
  Primer

SEQ ID NO: 93 - DNA, 43 bp, Artificial Sequence; identical to SEQ ID NO: 18
  Primer

SEQ ID NO: 94 - DNA, 44 bp, Artificial Sequence
  Primer
acaatttattgtattgggggatcatatgcttctacattcggtat

SEQ ID NO: 95 - DNA, 25 bp, Artificial Sequence
  Primer
tagaatttattgtattgggggatat

SEQ ID NO: 96 - DNA, 26 bp, Artificial Sequence
  Primer
gtagaatttattgtattgggggatat

SEQ ID NO: 97 - DNA, 25 bp, Artificial Sequence
  Primer
tacaatttattgtattgggggatat

SEQ ID NO: 98 - DNA, 26 bp, Artificial Sequence
  Primer
gtacaatttattgtattgggggatat

SEQ ID NO: 99 - DNA, 22 bp, Artificial Sequence
  Primer
ctaccatttgacgtaacaccac

SEQ ID NO: 100 - DNA, 23 bp, Artificial Sequence
  Primer
tctaccatttgacgtaacaccac

SEQ ID NO: 101 - DNA, 23 bp, Artificial Sequence
  Primer
tgtaccatttgacgtaacaccac

SEQ ID NO: 102 - DNA, 42 bp, Artificial Sequence; identical to SEQ ID NO: 53
  Primer